European Patent Application EP 4 778 942 A1, published July 22, 2026. Title: 一种广谱甲型流感疫苗免疫原组合物及应用. Applicant: 复旦大学. The sequence listing filed with the application follows.

SEQUENCE LISTING (52 sequences)

SEQ ID NO: 1 - protein, 185 aa, influenza virus
GLFGAIAGFIENGWEGLIDGWYGFRHQNAQGEGTAADYKSTQSAIDQITGKLNRLIEKTNQQFELIDNEFNEVEKQIGNVIRWTRDSITEVWSYNAELLVAMENQHTIDLADSEMDKLYERVKRQLRENAEEDGTGCFEIFHKCDDDCMASIRHNTYDHSKYREEAMQNRIQIDPVKLSSGYKDV

SEQ ID NO: 2 - DNA, 555 bp, influenza virus
  source 1..555: mol_type = genomic DNA
ggcctttttggagcaatcgctggattcattgaaaatgggtgggagggcctcatcgacgggtggtacggattcaggcaccaaaacgcccagggagaagggaccgcagctgactacaagtcaacacagtcagctattgatcagattaccgggaagctgaatagactgattgaaaagaccaaccagcagttcgagctgatcgataacgagtttaacgaggtcgaaaagcagataggaaatgtaatcaggtggacacgcgattctatcaccgaagtctggtcctacaatgccgagctgctggttgcaatggagaaccaacacactatcgaccttgccgattccgaaatggacaaactgtatgaacgcgtgaagcggcagctcagggaaaacgctgaggaagacggtaccggctgtttcgaaattttccacaagtgcgatgatgactgtatggccagcatcaggcacaacacctacgatcattccaagtatagagaggaggccatgcagaaccggattcagatcgatccagtgaaactgtcatccggctacaaggacgtg

SEQ ID NO: 3 - protein, 46 aa, Artificial sequence
DKIREVPEGWLIFVAEREELYVRVRNGFRKVLLEARTALPRGTGNE

SEQ ID NO: 4 - DNA, 138 bp, Artificial sequence
  source 1..138: mol_type = other DNA
gacaagatcagggaggtgcctgagggctggctcatcttcgtggccgagcgggaggagctgtacgtgcgggtgagaaacggcttcagaaaggtgctcttagaagcccggacagccctgccacggggcacaggcaacgag

SEQ ID NO: 5 - protein, 27 aa, Artificial sequence
GYIPEAPRDGQAYVRKDGEWVLLSTFL

SEQ ID NO: 6 - DNA, 81 bp, Artificial sequence
  source 1..81: mol_type = other DNA
ggatacattccagaggcccccagagacggacaggcttatgtgagaaaggacggagagtgggtgctgctgagtacatttctg

SEQ ID NO: 7 - protein, 49 aa, Artificial sequence
IINETADDIVYRLTVIIDDRYESLKNLITLRADRLEMIINDNVSTILAS

SEQ ID NO: 8 - DNA, 147 bp, Artificial sequence
  source 1..147: mol_type = other DNA
atcatcaacgagactgctgacgacatcgtgtaccgtctgaccgtgatcatcgacgaccgctacgagtccctgaagaacctgatcaccctgcgtgctgaccgtctggaaatgattatcaacgacaacgtgtccaccatcctggcttcc

SEQ ID NO: 9 - protein, 19 aa, Artificial sequence
EELLSKNYHLENEVARLKK

SEQ ID NO: 10 - DNA, 57 bp, Artificial sequence
  source 1..57: mol_type = other DNA
gaagaattgctttcgaaaaattatcacttggaaaatgaggttgccagattaaagaaa

SEQ ID NO: 11 - protein, 990 aa, Artificial sequence
MDVNPTLLFLKVPAQNAISTTFPYTGDPPYSHGTGTGYTMDTVNRTHQYSEKGKWTTNTETGAPQLNPIDGPLPEDNEPSGYAQHFQRKRRVRDNMTKKMVTQRTIGKKKQRLNKRGYLIRALTLNTMTKDAERGKLKRRAIATPGMQIRGFVYFVETLARSICEKLEQSGLPVGGNEKKAKLANVVRKMMTNSQDTEISFTITGDNTKWNENQNPRMFLAMITYITKNQPEWFRNILSIAPIMFSNKMARLGKGYMFESKRMKLRTQIPAEMLASIDLKYFNESTKKKIEKIRPLLIDGTASLSPGMMMGMFNMLSTVLGVSILNLGQKKYTKTTYWWDGLQSSDDFALIVNAPNHEGIQAGVDRFYRTCKLVGINMSKKKSYINKTGTFEFTSFFYRYGFVANFSMELPSFGVSGVNESADMSIGVTVIKNNMINNDLGPATAQMALQLFIKDYRYTYRCHRGDTQIQTRRSFELKKLWDQTQSKAGLLVSDGGPNLYNIRNLHIPEVCLKWELMDEDYRGRLCNPLNPFVSHKEIESVNNAVVMPAHGPAKSMEYDAVATTHSWIPKRNRSILNTSQRGILEDEQMYQKCCNLFEKFFPSSSYRRPVGISSMVEAMVSRARIDARIDFESGRIKKEEFSEIMKICSTIEELRRQKGGGGSGGGGSMRRNYFTAEVSHCRATEYIMKGVYINTALLNASCAAMDDFQLIPMISKCRTKEGRRKTNLYGFIIKGRSHLRNDTDVVNFVSMEFSLTDPRLEMFLYVRTNGTSKIKMKWGMEMRRCLLQSLQQIESMIEAESSVKEKDMTKEFFENKSETWPIGESPKGVEEGSIGKVCRTLLAKSVFNFDLGGLYEAIEECLINDPWVLLNASWFNSFLTHALKGSGGSGMTKITLSPQNFRIQKQETTLLKEKSTEKNSLAKSILAVKNHFIELRSKLSERFISHKNTESSATHFHRGSASEGRAVLTNKVVKDFMLQTLNDIDIRGSA

SEQ ID NO: 12 - DNA, 2970 bp, Artificial sequence
  source 1..2970: mol_type = other DNA
atggacgtgaaccccaccctgctgtttctgaaggtgcccgctcagaacgccatctccaccacattcccctacaccggcgaccctccttactcccatggcacaggaaccggctacaccatggacaccgtgaacagaacccaccagtacagcgagaaaggcaaatggaccaccaacaccgaaaccggcgcccctcagctgaaccctatcgatggacccctgcccgaagacaacgaaccctcaggatacgcccagcacttccagagaaaaagaagagtgagagacaacatgaccaaaaagatggtgacccagagaaccatcggcaagaagaaacagagactgaacaagagaggatacctgatcagagccctgaccctgaacaccatgaccaaggacgccgagagaggcaagctgaagagaagagccatcgccacccccggaatgcagatcagaggattcgtgtacttcgtggagaccctggccagaagcatctgcgaaaagctggagcagagcggactgccagtgggaggaaacgaaaaaaaggccaagctggccaacgtggtgagaaagatgatgaccaacagccaggacaccgagatcagcttcaccatcaccggcgacaacaccaagtggaacgagaaccagaaccccagaatgttcctggccatgatcacctacatcaccaagaaccagcccgagtggttcagaaacatcctgagcatcgcccccatcatgttcagcaacaagatggccagactgggcaagggctacatgttcgagagcaagagaatgaagctgagaacccagatccccgccgagatgctggccagcatcgacctgaagtacttcaacgagagcaccaagaagaagatcgagaagatcagacccctgctgatcgacggcaccgccagcctgagccccggcatgatgatgggcatgttcaacatgctgagcaccgtgctgggcgtgagcatcctgaacctgggccagaagaagtacaccaagaccacctactggtgggacggcctgcagagcagcgacgacttcgccctgatcgtgaacgcccccaaccacgagggcatccaggccggcgtggacagattctacagaacctgcaagctggtgggcatcaacatgagcaagaagaagagctacatcaacaagaccggcaccttcgagttcaccagcttcttctacagatacggcttcgtggccaacttcagcatggagctgcccagcttcggcgtgagcggcgtgaacgagagcgccgacatgagcatcggcgtgaccgtgatcaagaacaacatgatcaacaacgacctgggccccgccaccgcccagatggccctgcagctgttcatcaaggactacagatacacctacagatgccacagaggcgacacccagatccagaccagaagaagcttcgagctgaagaagctgtgggaccagacccagagcaaggccggcctgctggtgagcgacggcggccccaacctgtacaacatcagaaacctgcacatccccgaggtgtgcctgaagtgggagctgatggacgaggactacagaggcagactgtgcaaccccctgaaccccttcgtgagccacaaggagatcgagagcgtgaacaacgccgtggtgatgcccgcccacggccccgccaagagcatggagtacgacgccgtggccaccacccacagctggattcctaagagaaacagaagcatcctgaacaccagccagagaggcatcctggaggacgagcagatgtaccagaagtgctgcaacctgttcgagaagttcttccccagcagcagctacagaagacccgtgggcatcagcagcatggtggaggccatggtgagcagagccagaatcgacgccagaatcgacttcgagagcggcagaatcaagaaggaggagttcagcgagatcatgaagatctgcagcaccatcgaggagctgagaagacagaagggcggcggcggcagcggcggcggcggcagcatgagaagaaactacttcaccgccgaggtgagccactgcagagccaccgagtacatcatgaagggcgtgtacatcaacaccgccctgctgaacgccagctgcgccgccatggacgacttccagctgatccccatgatcagcaagtgcagaaccaaggagggcagaagaaagaccaacctgtacggcttcatcatcaagggcagaagccacctgagaaacgacaccgacgtggtgaacttcgtgagcatggagttcagcctgaccgaccccagactggagatgttcctgtacgtgagaaccaacggcaccagcaagatcaagatgaagtggggcatggagatgagaagatgcctgctgcagagcctgcagcagatcgagagcatgatcgaggccgagagcagcgtgaaggagaaggacatgaccaaggagttcttcgagaacaagagcgagacctggcccatcggcgagagccccaagggcgtggaggagggcagcatcggcaaggtgtgcagaaccctgctggccaagagcgtgttcaacttcgacctgggcggcctgtacgaggccatcgaggagtgcctgatcaacgacccctgggtgctgctgaacgccagctggttcaacagcttcctgacccacgccctgaagggcagcggcggcagcggcatgaccaagatcaccctgagcccccagaacttcagaatccagaagcaggagaccaccctgctgaaggagaagagcaccgagaagaacagcctggccaagagcatcctggccgtgaagaaccacttcatcgagctgagaagcaagctgagcgagagattcatcagccacaagaacaccgagagcagcgccacccacttccacagaggcagcgccagcgagggcagagccgtgctgaccaacaaggtggtgaaggacttcatgctgcagaccctgaacgacatcgacatcagaggcagcgcc

SEQ ID NO: 13 - protein, 24 aa, Artificial sequence
SLLTEVETPIRNEWGCRCNGSSDP

SEQ ID NO: 14 - DNA, 72 bp, Artificial sequence
  source 1..72: mol_type = other DNA
tccctcctgaccgaggtggagacacctatccggaacgagtgggggtgtagatgcaacggcagcagcgaccca

SEQ ID NO: 15 - protein, 24 aa, Artificial sequence
SLLTEVETPIRNEWGCRCNDSSDP

SEQ ID NO: 16 - DNA, 72 bp, Artificial sequence
  source 1..72: mol_type = other DNA
agcctcctcacagaggtggagacaccaatcaggaacgagtggggatgcagatgcaacgactctagcgaccca

SEQ ID NO: 17 - protein, 24 aa, Artificial sequence
SLLTEVETPTRTGWECNCSGSSEP

SEQ ID NO: 18 - DNA, 72 bp, Artificial sequence
  source 1..72: mol_type = other DNA
agtctcctcacagaggtggagacacctaccaggaccggctgggagtgcaactgctctggcagctctgagcca

SEQ ID NO: 19 - protein, 24 aa, Artificial sequence
SLLTEVETPTRNEWECKCSDSSDP

SEQ ID NO: 20 - DNA, 72 bp, Artificial sequence
  source 1..72: mol_type = other DNA
tctctcctcacagaggtggagacacctacaagaaacgagtgggagtgcaagtgctccgactcttccgaccca

SEQ ID NO: 21 - protein, 105 aa, Artificial sequence
SLLTEVETPIRNEWGCRCNGSSDPAAASLLTEVETPIRNEWGCRCNDSSDPAAASLLTEVETPTRTGWECNCSGSSEPAAASLLTEVETPTRNEWECKCSDSSDP

SEQ ID NO: 22 - DNA, 315 bp, Artificial sequence
  source 1..315: mol_type = other DNA
tccctcctgaccgaggtggagacacctatccggaacgagtgggggtgtagatgcaacggcagcagcgacccagctgccgcaagcctcctcacagaggtggagacaccaatcaggaacgagtggggatgcagatgcaacgactctagcgacccagctgccgcaagtctcctcacagaggtggagacacctaccaggaccggctgggagtgcaactgctctggcagctctgagccagctgccgcttctctcctcacagaggtggagacacctacaagaaacgagtgggagtgcaagtgctccgactcttccgaccca

SEQ ID NO: 23 - protein, 213 aa, Artificial sequence
SLLTEVETPIRNEWGCRCNGSSDPAAASLLTEVETPIRNEWGCRCNDSSDPAAASLLTEVETPTRTGWECNCSGSSEPAAASLLTEVETPTRNEWECKCSDSSDPAAASLLTEVETPIRNEWGCRCNGSSDPAAASLLTEVETPIRNEWGCRCNDSSDPAAASLLTEVETPTRTGWECNCSGSSEPAAASLLTEVETPTRNEWECKCSDSSDP

SEQ ID NO: 24 - DNA, 639 bp, Artificial sequence
  source 1..639: mol_type = other DNA
tccctcctgaccgaggtggagacacctatccggaacgagtgggggtgtagatgcaacggctcttctgaccccgccgccgcttccctcctcacagaggtggagacccctatcaggaacgagtggggttgcagatgcaacgactctagcgacccagccgccgcttctctcctgaccgaggtggagacaccaacaagaaccggctgggagtgcaactgctctggctcttctgagccagctgccgcttccctcctgaccgaggtggagacacctacaagaaacgagtgggagtgcaagtgctccgactctagcgaccccgccgccgcttccctgctcacagaggtggagacaccaatccggaacgagtggggttgtagatgcaacggcagcagcgacccagctgccgcaagcctcctcacagaggtggagacaccaatcaggaacgagtggggatgcagatgcaacgactctagcgacccagctgccgcaagtctcctcacagaggtggagacacctaccaggaccggctgggagtgcaactgctctggcagctctgagccagctgccgcttctctcctcacagaggtggagacacctacaagaaacgagtgggagtgcaagtgctccgactcttccgaccca

SEQ ID NO: 25 - protein, 450 aa, Artificial sequence
SLLTEVETPIRNEWGCRCNGSSDPAAASLLTEVETPIRNEWGCRCNDSSDPAAASLLTEVETPTRTGWECNCSGSSEPAAASLLTEVETPTRNEWECKCSDSSDPAAASLLTEVETPIRNEWGCRCNGSSDPAAASLLTEVETPIRNEWGCRCNDSSDPAAASLLTEVETPTRTGWECNCSGSSEPAAASLLTEVETPTRNEWECKCSDSSDPSAPGTPGLFGAIAGFIENGWEGLIDGWYGFRHQNAQGEGTAADYKSTQSAIDQITGKLNRLIEKTNQQFELIDNEFNEVEKQIGNVIRWTRDSITEVWSYNAELLVAMENQHTIDLADSEMDKLYERVKRQLRENAEEDGTGCFEIFHKCDDDCMASIRHNTYDHSKYREEAMQNRIQIDPVKLSSGYKDVDKIREVPEGWLIFVAEREELYVRVRNGFRKVLLEARTALPRGTGNE

SEQ ID NO: 26 - DNA, 1350 bp, Artificial sequence
  source 1..1350: mol_type = other DNA
tccctcctgaccgaggtggagacacctatccggaacgagtgggggtgtagatgcaacggctcttctgaccccgccgccgcttccctcctcacagaggtggagacccctatcaggaacgagtggggttgcagatgcaacgactctagcgacccagccgccgcttctctcctgaccgaggtggagacaccaacaagaaccggctgggagtgcaactgctctggctcttctgagccagctgccgcttccctcctgaccgaggtggagacacctacaagaaacgagtgggagtgcaagtgctccgactctagcgaccccgccgccgcttccctgctcacagaggtggagacaccaatccggaacgagtggggttgtagatgcaacggcagcagcgacccagctgccgcaagcctcctcacagaggtggagacaccaatcaggaacgagtggggatgcagatgcaacgactctagcgacccagctgccgcaagtctcctcacagaggtggagacacctaccaggaccggctgggagtgcaactgctctggcagctctgagccagctgccgcttctctcctcacagaggtggagacacctacaagaaacgagtgggagtgcaagtgctccgactcttccgacccaagcgccccaggcacacctggcctttttggagcaatcgctggattcattgaaaatgggtgggagggcctcatcgacgggtggtacggattcaggcaccaaaacgcccagggagaagggaccgcagctgactacaagtcaacacagtcagctattgatcagattaccgggaagctgaatagactgattgaaaagaccaaccagcagttcgagctgatcgataacgagtttaacgaggtcgaaaagcagataggaaatgtaatcaggtggacacgcgattctatcaccgaagtctggtcctacaatgccgagctgctggttgcaatggagaaccaacacactatcgaccttgccgattccgaaatggacaaactgtatgaacgcgtgaagcggcagctcagggaaaacgctgaggaagacggtaccggctgtttcgaaattttccacaagtgcgatgatgactgtatggccagcatcaggcacaacacctacgatcattccaagtatagagaggaggccatgcagaaccggattcagatcgatccagtgaaactgtcatccggctacaaggacgtggacaagatcagggaggtgcctgagggctggctcatcttcgtggccgagcgggaggagctgtacgtgcgggtgagaaacggcttcagaaaggtgctcttagaagcccggacagccctgccacggggcacaggcaacgag

SEQ ID NO: 27 - protein, 328 aa, Artificial sequence
SLLTEVETPIRNEWGCRCNGSSDPAAASLLTEVETPIRNEWGCRCNDSSDPAAASLLTEVETPTRTGWECNCSGSSEPAAASLLTEVETPTRNEWECKCSDSSDPSAPGTPGLFGAIAGFIENGWEGLIDGWYGFRHQNAQGEGTAADYKSTQSAIDQITGKLNRLIEKTNQQFELIDNEFNEVEKQIGNVIRWTRDSITEVWSYNAELLVAMENQHTIDLADSEMDKLYERVKRQLRENAEEDGTGCFEIFHKCDDDCMASIRHNTYDHSKYREEAMQNRIQIDPVKLSSGYKDVLETGGGYIPEAPRDGQAYVRKDGEWVLLSTFL

SEQ ID NO: 28 - DNA, 984 bp, Artificial sequence
  source 1..984: mol_type = other DNA
tccctcctgaccgaggtggagacacctatccggaacgagtgggggtgtagatgcaacggcagcagcgacccagctgccgcaagcctcctcacagaggtggagacaccaatcaggaacgagtggggatgcagatgcaacgactctagcgacccagctgccgcaagtctcctcacagaggtggagacacctaccaggaccggctgggagtgcaactgctctggcagctctgagccagctgccgcttctctcctcacagaggtggagacacctacaagaaacgagtgggagtgcaagtgctccgactcttccgacccaagcgccccaggcacacctggcctttttggagcaatcgctggattcattgaaaatgggtgggagggcctcatcgacgggtggtacggattcaggcaccaaaacgcccagggagaagggaccgcagctgactacaagtcaacacagtcagctattgatcagattaccgggaagctgaatagactgattgaaaagaccaaccagcagttcgagctgatcgataacgagtttaacgaggtcgaaaagcagataggaaatgtaatcaggtggacacgcgattctatcaccgaagtctggtcctacaatgccgagctgctggttgcaatggagaaccaacacactatcgaccttgccgattccgaaatggacaaactgtatgaacgcgtgaagcggcagctcagggaaaacgctgaggaagacggtaccggctgtttcgaaattttccacaagtgcgatgatgactgtatggccagcatcaggcacaacacctacgatcattccaagtatagagaggaggccatgcagaaccggattcagatcgatccagtgaaactgtcatccggctacaaggacgtgctcgagaccggcggcggatacattccagaggcccccagagacggacaggcttatgtgagaaaggacggagagtgggtgctgctgagtacatttctg

SEQ ID NO: 29 - protein, 331 aa, Artificial sequence
SLLTEVETPIRNEWGCRCNGSSDPAAASLLTEVETPIRNEWGCRCNDSSDPAAASLLTEVETPTRTGWECNCSGSSEPAAASLLTEVETPTRNEWECKCSDSSDPSAPGTPCTGLFGAIAGFIEGGWTGMIDGWYGYHHQNEQGSGYAADQKSTQNAINGITNKVNSVIEKMNIQFTAVGKEFNKLEKRMENLNKKVDDGFLDIWTYNAELLVLLENERTLDFHDSNVKNLYEKVKSQLKNNAKEIGNGCFEFYHKCDNECMESVRNGTYDYPKYSEESKLNREKVDGVKLESMGIYQILETGGGYIPEAPRDGQAYVRKDGEWVLLSTFL

SEQ ID NO: 30 - DNA, 993 bp, Artificial sequence
  source 1..993: mol_type = other DNA
tccctcctgaccgaggtggagacacctatccggaacgagtgggggtgtagatgcaacggcagcagcgacccagctgccgcaagcctcctcacagaggtggagacaccaatcaggaacgagtggggatgcagatgcaacgactctagcgacccagctgccgcaagtctcctcacagaggtggagacacctaccaggaccggctgggagtgcaactgctctggcagctctgagccagctgccgcttctctcctcacagaggtggagacacctacaagaaacgagtgggagtgcaagtgctccgactcttccgacccaagcgccccaggcacaccttgtacaggcctgttcggcgcgatcgcgggcttcatcgaaggcggctggaccggcatgatcgatggctggtacggctaccaccaccagaacgaacagggcagcggctacgcggctgatcagaaaagcacccagaacgcgatcaacggcatcaccaacaaagttaacagcgttatcgaaaaaatgaacatccagttcaccgcggttggtaaagaattcaacaaactggaaaagcgtatggaaaacctgaacaaaaaagttgatgatggcttcctggatatctggacctacaacgcggaactgctggttctgctggaaaacgaacgtaccctggatttccacgatagcaacgtgaaaaacctgtacgaaaaagttaaaagccagctgaaaaacaacgcgaaagaaatcggtaacggctgcttcgaattctaccacaaatgcgataacgaatgtatggaaagcgttcgtaacggtacttatgattaccctaagtattccgaagaatctaaactgaaccgtgaaaaagttgacggcgtcaaattagaatctatgggtatctatcagatcctcgagaccggcggcggatacattccagaggcccccagagacggacaggcttatgtgagaaaggacggagagtgggtgctgctgagtacatttctg

SEQ ID NO: 31 - protein, 329 aa, Artificial sequence
SLLTEVETPIRNEWGCRCNGSSDPAAASLLTEVETPIRNEWGCRCNDSSDPAAASLLTEVETPTRTGWECNCSGSSEPAAASLLTEVETPTRNEWECKCSDSSDPSAPGTPCTGLFGAIAGFIENGWEGMIDGWYGFRHQNSEGTGQAADLKSTQAAIDQINGKLNRVIEKTNEKFHQIEKEFSEVEGRIQDLEKYVEDTKIDLWSYNAELLVALENQHTIDLTDSEMNKLFEKTRRQLRENAEDMGNGCFKIYHKCDNACIESIRNGTYDHDVYRDEALNNRFQIKGVELKSGYKDLETGGGYIPEAPRDGQAYVRKDGEWVLLSTFL

SEQ ID NO: 32 - DNA, 987 bp, Artificial sequence
  source 1..987: mol_type = other DNA
tccctcctgaccgaggtggagacacctatccggaacgagtgggggtgtagatgcaacggcagcagcgacccagctgccgcaagcctcctcacagaggtggagacaccaatcaggaacgagtggggatgcagatgcaacgactctagcgacccagctgccgcaagtctcctcacagaggtggagacacctaccaggaccggctgggagtgcaactgctctggcagctctgagccagctgccgcttctctcctcacagaggtggagacacctacaagaaacgagtgggagtgcaagtgctccgactcttccgacccaagcgccccaggcacaccttgtacaggcctgttcggggcgatagcaggcttcattgaaaacgggtgggagggtatgattgatggctggtacggcttccgtcaccagaacagcgaaggtaccggccaggcggcggatctgaaaagcacccaggcggcgatcgatcagatcaacggtaaactgaaccgtgttatcgaaaaaaccaacgaaaaattccaccagatcgaaaaagaattcagcgaagttgaaggccgtatccaggatctggaaaaatacgttgaagataccaaaatcgatctgtggagctacaacgcggaactgctggttgcgctggaaaaccagcacacgatcgatctgaccgatagcgaaatgaacaaactgttcgaaaaaacccgtcgtcagctgcgtgaaaacgcggaagatatgggtaacggttgcttcaaaatctaccacaaatgcgataacgcgtgcatcgaaagcatccgtaacggcacctacgatcacgatgtttaccgtgatgaagcgctgaacaaccgtttccagatcaaaggcgttgaactgaaaagcggctacaaagatctcgagaccggcggcggatacattccagaggcccccagagacggacaggcttatgtgagaaaggacggagagtgggtgctgctgagtacatttctg

SEQ ID NO: 33 - protein, 274 aa, Artificial sequence
SLLTEVETPIRNEWGCRCNGSSDPAAASLLTEVETPIRNEWGCRCNDSSDPRTSAPGGLFGAIAGFIENGWEGLIDGWYGFRHQNAQGEGTAADYKSTQSAIDQITGKLNRLIEKTNQQFELIDNEFNEVEKQIGNVIRWTRDSITEVWSYNAELLVAMENQHTIDLADSEMDKLYERVKRQLRENAEEDGTGCFEIFHKCDDDCMASIRHNTYDHSKYREEAMQNRIQIDPVKLSSGYKDVLETGGGYIPEAPRDGQAYVRKDGEWVLLSTFL

SEQ ID NO: 34 - DNA, 822 bp, Artificial sequence
  source 1..822: mol_type = other DNA
tccctcctgaccgaggtggagacacctatccggaacgagtgggggtgtagatgcaacggcagcagcgacccagctgccgcaagcctcctcacagaggtggagacaccaatcaggaacgagtggggatgcagatgcaacgactctagcgacccacgtacgagcgccccaggcggcctttttggagcaatcgctggattcattgaaaatgggtgggagggcctcatcgacgggtggtacggattcaggcaccaaaacgcccagggagaagggaccgcagctgactacaagtcaacacagtcagctattgatcagattaccgggaagctgaatagactgattgaaaagaccaaccagcagttcgagctgatcgataacgagtttaacgaggtcgaaaagcagataggaaatgtaatcaattggacacgcgattctatcaccgaagtctggtcctacaatgccgagctgctggttgcaatggagaaccaacacactatcgaccttgccgattccgaaatggacaaactgtatgaacgcgtgaagcggcagctcagggaaaacgctgaggaagacggtaccggctgtttcgaaattttccacaagtgcgatgatgactgtatggccagcatcaggaataacacctacgatcattccaagtatagagaggaggccatgcagaaccggattcagatcgatccagtgaaactgtcatccggctacaaggacgtgctcgagaccggcggcggatacattccagaggcccccagagacggacaggcttatgtgagaaaggacggagagtgggtgctgctgagtacatttctg

SEQ ID NO: 35 - protein, 296 aa, Artificial sequence
SLLTEVETPIRNEWGCRCNGSSDPAAASLLTEVETPIRNEWGCRCNDSSDPAAASLLTEVETPTRTGWECNCSGSSEPAAASLLTEVETPTRNEWECKCSDSSDPSAPGTPGLFGAIAGFIENGWEGLIDGWYGFRHQNAQGEGTAADYKSTQSAIDQITGKLNRLIEKTNQQFELIDNEFNEVEKQIGNVIRWTRDSITEVWSYNAELLVAMENQHTIDLADSEMDKLYERVKRQLRENAEEDGTGCFEIFHKCDDDCMASIRHNTYDHSKYREEAMQNRIQIDPVKLSSGYKDV

SEQ ID NO: 36 - DNA, 888 bp, Artificial sequence
  source 1..888: mol_type = other DNA
tccctcctgaccgaggtggagacacctatccggaacgagtgggggtgtagatgcaacggcagcagcgacccagctgccgcaagcctcctcacagaggtggagacaccaatcaggaacgagtggggatgcagatgcaacgactctagcgacccagctgccgcaagtctcctcacagaggtggagacacctaccaggaccggctgggagtgcaactgctctggcagctctgagccagctgccgcttctctcctcacagaggtggagacacctacaagaaacgagtgggagtgcaagtgctccgactcttccgacccaagcgccccaggcacacctggcctttttggagcaatcgctggattcattgaaaatgggtgggagggcctcatcgacgggtggtacggattcaggcaccaaaacgcccagggagaagggaccgcagctgactacaagtcaacacagtcagctattgatcagattaccgggaagctgaatagactgattgaaaagaccaaccagcagttcgagctgatcgataacgagtttaacgaggtcgaaaagcagataggaaatgtaatcaggtggacacgcgattctatcaccgaagtctggtcctacaatgccgagctgctggttgcaatggagaaccaacacactatcgaccttgccgattccgaaatggacaaactgtatgaacgcgtgaagcggcagctcagggaaaacgctgaggaagacggtaccggctgtttcgaaattttccacaagtgcgatgatgactgtatggccagcatcaggcacaacacctacgatcattccaagtatagagaggaggccatgcagaaccggattcagatcgatccagtgaaactgtcatccggctacaaggacgtg

SEQ ID NO: 37 - protein, 217 aa, Artificial sequence
GLFGAIAGFIENGWEGLIDGWYGFRHQNAQGEGTAADYKSTQSAIDQITGKLNRLIEKTNQQFELIDNEFNEVEKQIGNVIRWTRDSITEVWSYNAELLVAMENQHTIDLADSEMDKLYERVKRQLRENAEEDGTGCFEIFHKCDDDCMASIRHNTYDHSKYREEAMQNRIQIDPVKLSSGYKDVLETGGGYIPEAPRDGQAYVRKDGEWVLLSTFL

SEQ ID NO: 38 - DNA, 651 bp, Artificial sequence
  source 1..651: mol_type = other DNA
ggcctttttggagcaatcgctggattcattgaaaatgggtgggagggcctcatcgacgggtggtacggattcaggcaccaaaacgcccagggagaagggaccgcagctgactacaagtcaacacagtcagctattgatcagattaccgggaagctgaatagactgattgaaaagaccaaccagcagttcgagctgatcgataacgagtttaacgaggtcgaaaagcagataggaaatgtaatcaggtggacacgcgattctatcaccgaagtctggtcctacaatgccgagctgctggttgcaatggagaaccaacacactatcgaccttgccgattccgaaatggacaaactgtatgaacgcgtgaagcggcagctcagggaaaacgctgaggaagacggtaccggctgtttcgaaattttccacaagtgcgatgatgactgtatggccagcatcaggcacaacacctacgatcattccaagtatagagaggaggccatgcagaaccggattcagatcgatccagtgaaactgtcatccggctacaaggacgtgctcgagaccggcggcggatacattccagaggcccccagagacggacaggcttatgtgagaaaggacggagagtgggtgctgctgagtacatttctg

SEQ ID NO: 39 - protein, 347 aa, Artificial sequence
SLLTEVETPIRNEWGCRCNGSSDPAAASLLTEVETPIRNEWGCRCNDSSDPAAASLLTEVETPTRTGWECNCSGSSEPAAASLLTEVETPTRNEWECKCSDSSDPKTACTSAPGTPGLFGAIAGFIENGWEGLIDGWYGFRHQNAQGEGTAADYKSTQSAIDQITGKLNRLIEKTNQQFELIDNEFNEVEKQIGNVIRWTRDSITEVWSYNAELLVAMENQHTIDLADSEMDKLYERVKRQLRENAEEDGTGCFEIFHKCDDDCMASIRHNTYDHSKYREEAMQNRIQIDPVKLSSGYKDVDKIREVPEGWLIFVAEREELYVRVRNGFRKVLLEARTALPRGTGNE

SEQ ID NO: 40 - DNA, 1041 bp, Artificial sequence
  source 1..1041: mol_type = other DNA
tccctcctgaccgaggtggagacacctatccggaacgagtgggggtgtagatgcaacggcagcagcgacccagctgccgcaagcctcctcacagaggtggagacaccaatcaggaacgagtggggatgcagatgcaacgactctagcgacccagctgccgcaagtctcctcacagaggtggagacacctaccaggaccggctgggagtgcaactgctctggcagctctgagccagctgccgcttctctcctcacagaggtggagacacctacaagaaacgagtgggagtgcaagtgctccgactcttccgacccaaagaccgcttgtacaagcgccccaggcacacctggcctttttggagcaatcgctggattcattgaaaatgggtgggagggcctcatcgacgggtggtacggattcaggcaccaaaacgcccagggagaagggaccgcagctgactacaagtcaacacagtcagctattgatcagattaccgggaagctgaatagactgattgaaaagaccaaccagcagttcgagctgatcgataacgagtttaacgaggtcgaaaagcagataggaaatgtaatcaggtggacacgcgattctatcaccgaagtctggtcctacaatgccgagctgctggttgcaatggagaaccaacacactatcgaccttgccgattccgaaatggacaaactgtatgaacgcgtgaagcggcagctcagggaaaacgctgaggaagacggtaccggctgtttcgaaattttccacaagtgcgatgatgactgtatggccagcatcaggcacaacacctacgatcattccaagtatagagaggaggccatgcagaaccggattcagatcgatccagtgaaactgtcatccggctacaaggacgtggacaagatcagggaggtgcctgagggctggctcatcttcgtggccgagcgggaggagctgtacgtgcgggtgagaaacggcttcagaaaggtgctcttagaagcccggacagccctgccacggggcacaggcaacgag

SEQ ID NO: 41 - DNA, 469 bp, Artificial sequence
  source 1..469: mol_type = other DNA
gagggcccggaaacctggccctgtcttcttgacgagcattcctaggggtctttcccctctcgccaaaggaatgcaaggtctgttgaatgtcgtgaaggaagcagttcctctggaagcttcttgaagacaaacaacgtctgtagcgaccctttgcaggcagcggaaccccccacctggcgacaggtgcctctgcggccaaaagccacgtgtataagatacacctgcaaaggcggcacaaccccagtgccacgttgtgagttggatagttgtggaaagagtcaaatggctctcctcaagcgtattcaacaaggggctgaaggatgcccagaaggtaccccattgtatgggatctgatctggggcctcggtgcacatgctttacatgtgtttagtcgaggttaaaaaaacgtctaggccccccgaaccacggggacgtggttttcctttgaaaaacacgatgataagccacc

SEQ ID NO: 42 - DNA, 4927 bp, Artificial sequence
  source 1..4927: mol_type = other DNA
tccctcctgaccgaggtggagacacctatccggaacgagtgggggtgtagatgcaacggcagcagcgacccagctgccgcaagcctcctcacagaggtggagacaccaatcaggaacgagtggggatgcagatgcaacgactctagcgacccagctgccgcaagtctcctcacagaggtggagacacctaccaggaccggctgggagtgcaactgctctggcagctctgagccagctgccgcttctctcctcacagaggtggagacacctacaagaaacgagtgggagtgcaagtgctccgactcttccgacccaagcgccccaggcacacctggcctttttggagcaatcgctggattcattgaaaatgggtgggagggcctcatcgacgggtggtacggattcaggcaccaaaacgcccagggagaagggaccgcagctgactacaagtcaacacagtcagctattgatcagattaccgggaagctgaatagactgattgaaaagaccaaccagcagttcgagctgatcgataacgagtttaacgaggtcgaaaagcagataggaaatgtaatcaattggacacgcgattctatcaccgaagtctggtcctacaatgccgagctgctggttgcaatggagaaccaacacactatcgaccttgccgattccgaaatggacaaactgtatgaacgcgtgaagcggcagctcagggaaaacgctgaggaagacggtaccggctgtttcgaaattttccacaagtgcgatgatgactgtatggccagcatcaggaataacacctacgatcattccaagtatagagaggaggccatgcagaaccggattcagatcgatccagtgaaactgtcatccggctacaaggacgtgctcgagaccggcggcggatacattccagaggcccccagagacggacaggcttatgtgagaaaggacggagagtgggtgctgctgagtacatttctggagggcccggaaacctggccctgtcttcttgacgagcattcctaggggtctttcccctctcgccaaaggaatgcaaggtctgttgaatgtcgtgaaggaagcagttcctctggaagcttcttgaagacaaacaacgtctgtagcgaccctttgcaggcagcggaaccccccacctggcgacaggtgcctctgcggccaaaagccacgtgtataagatacacctgcaaaggcggcacaaccccagtgccacgttgtgagttggatagttgtggaaagagtcaaatggctctcctcaagcgtattcaacaaggggctgaaggatgcccagaaggtaccccattgtatgggatctgatctggggcctcggtgcacatgctttacatgtgtttagtcgaggttaaaaaaacgtctaggccccccgaaccacggggacgtggttttcctttgaaaaacacgatgataagccaccatggacgtgaaccccaccctgctgtttctgaaggtgcccgctcagaacgccatctccaccacattcccctacaccggcgaccctccttactcccatggcacaggaaccggctacaccatggacaccgtgaacagaacccaccagtacagcgagaaaggcaaatggaccaccaacaccgaaaccggcgcccctcagctgaaccctatcgatggacccctgcccgaagacaacgaaccctcaggatacgcccagcacttccagagaaaaagaagagtgagagacaacatgaccaaaaagatggtgacccagagaaccatcggcaagaagaaacagagactgaacaagagaggatacctgatcagagccctgaccctgaacaccatgaccaaggacgccgagagaggcaagctgaagagaagagccatcgccacccccggaatgcagatcagaggattcgtgtacttcgtggagaccctggccagaagcatctgcgaaaagctggagcagagcggactgccagtgggaggaaacgaaaaaaaggccaagctggccaacgtggtgagaaagatgatgaccaacagccaggacaccgagatcagcttcaccatcaccggcgacaacaccaagtggaacgagaaccagaaccccagaatgttcctggccatgatcacctacatcaccaagaaccagcccgagtggttcagaaacatcctgagcatcgcccccatcatgttcagcaacaagatggccagactgggcaagggctacatgttcgagagcaagagaatgaagctgagaacccagatccccgccgagatgctggccagcatcgacctgaagtacttcaacgagagcaccaagaagaagatcgagaagatcagacccctgctgatcgacggcaccgccagcctgagccccggcatgatgatgggcatgttcaacatgctgagcaccgtgctgggcgtgagcatcctgaacctgggccagaagaagtacaccaagaccacctactggtgggacggcctgcagagcagcgacgacttcgccctgatcgtgaacgcccccaaccacgagggcatccaggccggcgtggacagattctacagaacctgcaagctggtgggcatcaacatgagcaagaagaagagctacatcaacaagaccggcaccttcgagttcaccagcttcttctacagatacggcttcgtggccaacttcagcatggagctgcccagcttcggcgtgagcggcgtgaacgagagcgccgacatgagcatcggcgtgaccgtgatcaagaacaacatgatcaacaacgacctgggccccgccaccgcccagatggccctgcagctgttcatcaaggactacagatacacctacagatgccacagaggcgacacccagatccagaccagaagaagcttcgagctgaagaagctgtgggaccagacccagagcaaggccggcctgctggtgagcgacggcggccccaacctgtacaacatcagaaacctgcacatccccgaggtgtgcctgaagtgggagctgatggacgaggactacagaggcagactgtgcaaccccctgaaccccttcgtgagccacaaggagatcgagagcgtgaacaacgccgtggtgatgcccgcccacggccccgccaagagcatggagtacgacgccgtggccaccacccacagctggattcctaagagaaacagaagcatcctgaacaccagccagagaggcatcctggaggacgagcagatgtaccagaagtgctgcaacctgttcgagaagttcttccccagcagcagctacagaagacccgtgggcatcagcagcatggtggaggccatggtgagcagagccagaatcgacgccagaatcgacttcgagagcggcagaatcaagaaggaggagttcagcgagatcatgaagatctgcagcaccatcgaggagctgagaagacagaagggcggcggcggcagcggcggcggcggcagcatgagaagaaactacttcaccgccgaggtgagccactgcagagccaccgagtacatcatgaagggcgtgtacatcaacaccgccctgctgaacgccagctgcgccgccatggacgacttccagctgatccccatgatcagcaagtgcagaaccaaggagggcagaagaaagaccaacctgtacggcttcatcatcaagggcagaagccacctgagaaacgacaccgacgtggtgaacttcgtgagcatggagttcagcctgaccgaccccagactggagatgttcctgtacgtgagaaccaacggcaccagcaagatcaagatgaagtggggcatggagatgagaagatgcctgctgcagagcctgcagcagatcgagagcatgatcgaggccgagagcagcgtgaaggagaaggacatgaccaaggagttcttcgagaacaagagcgagacctggcccatcggcgagagccccaagggcgtggaggagggcagcatcggcaaggtgtgcagaaccctgctggccaagagcgtgttcaacttcgacctgggcggcctgtacgaggccatcgaggagtgcctgatcaacgacccctgggtgctgctgaacgccagctggttcaacagcttcctgacccacgccctgaagggcagcggcggcagcggcatgaccaagatcaccctgagcccccagaacttcagaatccagaagcaggagaccaccctgctgaaggagaagagcaccgagaagaacagcctggccaagagcatcctggccgtgaagaaccacttcatcgagctgagaagcaagctgagcgagagattcatcagccacaagaacaccgagagcagcgccacccacttccacagaggcagcgccagcgagggcagagccgtgctgaccaacaaggtggtgaaggacttcatgctgcagaccctgaacgacatcgacatcagaggcagcgccgcggccgccaccatgatcagcctgatcgccgccctggccgtggactacgtgctgggcatggagaacgccatgccctggaacctgcccgccgacctggcctggttcaagcggaacaccctgaacaagcccgtgatcatgggcagacacacctgggagtccatcggcagacccctgcccggcagaaagaacatcatcctatcgtcccagccctccaccgacgaccgggtgacctgggtgaagagcgtggacgaggccatcgccgcctgcggcgacgtgcccgagatcatggtgatcggcggcggcagagtgatcgagcagttcctgcccaaggcccagaagctgtacctgacccacctggacgccgaggtggagggcgacacccacttccccgactacgagcccgacgactgggagtccgtgttcagcgagttccacgacgccgacgcccagaacagccactcctactgcttcgagatcctggagagaaggggcggcggcggctct

SEQ ID NO: 43 - protein, 164 aa, Artificial sequence
MISLIAALAVDYVLGMENAMPWNLPADLAWFKRNTLNKPVIMGRHTWESIGRPLPGRKNIILSSQPSTDDRVTWVKSVDEAIAACGDVPEIMVIGGGRVIEQFLPKAQKLYLTHLDAEVEGDTHFPDYEPDDWESVFSEFHDADAQNSHSYCFEILERRGGGGS

SEQ ID NO: 44 - DNA, 492 bp, Artificial sequence
  source 1..492: mol_type = other DNA
atgatcagcctgatcgccgccctggccgtggactacgtgctgggcatggagaacgccatgccctggaacctgcccgccgacctggcctggttcaagcggaacaccctgaacaagcccgtgatcatgggcagacacacctgggagtccatcggcagacccctgcccggcagaaagaacatcatcctatcgtcccagccctccaccgacgaccgggtgacctgggtgaagagcgtggacgaggccatcgccgcctgcggcgacgtgcccgagatcatggtgatcggcggcggcagagtgatcgagcagttcctgcccaaggcccagaagctgtacctgacccacctggacgccgaggtggagggcgacacccacttccccgactacgagcccgacgactgggagtccgtgttcagcgagttccacgacgccgacgcccagaacagccactcctactgcttcgagatcctggagagaaggggcggcggcggctct

SEQ ID NO: 45 - protein, 5 aa, Artificial sequence
GGGGS

SEQ ID NO: 46 - protein, 12 aa, Artificial sequence
GSAGSAAGSGEF

SEQ ID NO: 47 - protein, 5 aa, Artificial sequence
EAAAK

SEQ ID NO: 48 - protein, 16 aa, Artificial sequence
EFPKPSTPPGSSGGAP

SEQ ID NO: 49 - protein, 18 aa, Artificial sequence
KESGSVSSEQLAQFRSLD

SEQ ID NO: 50 - protein, 14 aa, Artificial sequence
EGKSSGSGSESKST

SEQ ID NO: 51 - protein, 1169 aa, Artificial sequence
MERIKELRNLMSQSRTREILTKTTVDHMAIIKKYTSGKWMMAMKYPITADKRITEMIPERNEQGQTLWSKMNDAGSDRVMVSPLAVTWWNRNGPVTSTVHYPKVYKTYFEKVERLKHGTFGPVHFRNQVKQLTITKEKKEELQDCKISPLMVAYMLERELVRKTRFLPVAGGTSSVYIEVLIVRRAAVSADPLASLLEMCHSGLRISSSFSFGGFTFKRTSGSSVKKEEEVLTGNLQTLKIRIVSGRDEQSIAEAIIVAMVFSPMHQLLRHFQKDAKVLFQNWGIEHIDNVMGMIGILPDMTPSTEMSVSIDRFLRVRDQRGNVLLSPEEVSETQGTEKLTITYSSSMMWEINGPESVLVNTYQWIIRNWEAVKIQWSQNPTMLYNKMEFEPFQSLVPKAIRSQYSGFVRTLFQQMRDVLGTFDTTQIIKLLPFAAAPPKQSRMQFSSLTVNVRGSGMRILVRGNSPVFNYNKTTKRLTVLGKDAGTLTEDPDEGTSGVESAVLRGFLILGKEDRRYGPALSINELSVMKRKRDSSILTDSQTATKRIRMAINGSGGSGMASQGTKRSYEQMETDGERQNATEIRASVGRMIGGIGRFYIQMCTELKLSDYEGRLIQNSLTIERMVLSAFDERRNKYLEEHPSAGKDPKKTGGPIYRRVDGKWMRELVLYDKEEIRRIWRQANNGEDATAGLTHIMIWHSNLNDATYQRTRALVRTGMDPRMCSLMQGSTLPRRSGAAGAAVKGVGTMVMELIRMIKRGINDRNFWRGENGRKTRVAYERMCNILKGKFQTAAQRAMMDQVRESRNPGNAEIEDLIFLARSALILRGSVAHKSCLPACVYGPAVASGYDFEKEGYSLVGIDPFKLLQNSQVYSLIRPNENPAHKSQLVWMACHSAAFEDLRVSSFIRGTKVIPRGKLSTRGVQIASNENMDTMDSSTLELRSRYWAIRTRSGGNTNQQRASAGQISVQPTFSVQRNLPFEKSTVMAAFTGNTEGRTSDMRAEIIRMMESAKPEEVSFQGRGVFELSDEKATNPIVPSFDMSNEGSYFFGDNAEEYDNGGGGSGGGGSGGGGSMSLLTEVETPIRNEWGCRCNDSSDPLVVAANIIGILHLILWILDRLFFKCIYRLFKHGLKRGPSTEGVPESMREEYRKEQQNAVDADDSHFVSIELE

SEQ ID NO: 52 - protein, 1147 aa, Artificial sequence
MDVNPTLLFLKVPAQNAISTTFPYTGDPPYSHGTGTGYTMDTVNRTHQYSEKGKWTTNTETGAPQLNPIDGPLPEDNEPSGYAQHFQRKRRVRDNMTKKMVTQRTIGKKKQRLNKRGYLIRALTLNTMTKDAERGKLKRRAIATPGMQIRGFVYFVETLARSICEKLEQSGLPVGGNEKKAKLANVVRKMMTNSQDTEISFTITGDNTKWNENQNPRMFLAMITYITKNQPEWFRNILSIAPIMFSNKMARLGKGYMFESKRMKLRTQIPAEMLASIDLKYFNESTKKKIEKIRPLLIDGTASLSPGMMMGMFNMLSTVLGVSILNLGQKKYTKTTYWWDGLQSSDDFALIVNAPNHEGIQAGVDRFYRTCKLVGINMSKKKSYINKTGTFEFTSFFYRYGFVANFSMELPSFGVSGVNESADMSIGVTVIKNNMINNDLGPATAQMALQLFIKDYRYTYRCHRGDTQIQTRRSFELKKLWDQTQSKAGLLVSDGGPNLYNIRNLHIPEVCLKWELMDEDYRGRLCNPLNPFVSHKEIESVNNAVVMPAHGPAKSMEYDAVATTHSWIPKRNRSILNTSQRGILEDEQMYQKCCNLFEKFFPSSSYRRPVGISSMVEAMVSRARIDARIDFESGRIKKEEFSEIMKICSTIEELRRQKGGGGSGGGGSGGGGSMRRNYFTAEVSHCRATEYIMKGVYINTALLNASCAAMDDFQLIPMISKCRTKEGRRKTNLYGFIIKGRSHLRNDTDVVNFVSMEFSLTDPRLEMFLYVRTNGTSKIKMKWGMEMRRCLLQSLQQIESMIEAESSVKEKDMTKEFFENKSETWPIGESPKGVEEGSIGKVCRTLLAKSVFNFDLGGLYEAIEECLINDPWVLLNASWFNSFLTHALKGSGGSGMSLLTEVETYVLSIVPSGPLKAEIAQRLEDVFAGKNTDLEALMEWLKTRPILSPLTKGILGFVFTLTVPSERGLQRRRFVQNALNGNGDPNNMDRAVKLYRKLKREITFHGAKEIALSYSAGALASCMGLIYNRMGAVTTEVAFGLVCATCEQIADSQHRSHRQMVTTTNPLIRHENRMVLASTTAKAMEQMAGSSEQAAEAMEVASQARQMVQAMRAIGTHPSSSTGLKDDLLENLQAYQKRMGVQMQRFK